European Patent Application EP 4 588 935 A1, published July 23, 2025. Title: MARKER AND METHOD FOR DETECTING INFLAMMATION-RELATED DISEASES. Applicant: BEIJING MDTK BIOLOGY TECHNOLOGY CO.LTD. The sequence listing filed with the application follows.

SEQUENCE LISTING (10 sequences)

SEQ ID NO: 1 - protein, 112 aa, synthetic construct
QVQLQQPGTELVKPGASVKLSCKASGYTFTNYWIHWVKQRPGQGLEWIGNTKPSNGDIHYNEKFRSKATLTVDKSSSTAYIQLSSLTSEDSAVYFCAVGYYWGQGTTLTVSS

SEQ ID NO: 2 - protein, 112 aa, synthetic construct
DIVMTQSPSSLTVTAGEKVTMSCKSSQSLLNSGNQKNYLTWYQQKPGQPPKMLIYWAYNRDSGVPDRFTGSGSGADFTLTISSVQAEDLAVYYCQNDYSYPLTFGAGTKLEL

SEQ ID NO: 3 - protein, 209 aa, synthetic construct
GVPAEGAFTEDFQGLRAEVETISKELELLDRELCQLLLEGLEGVLRDQLALRALEEALEQGQSLGPVEPLDGPAGAVLECLVLSSGMLVPELAIPVVYLLGALTMLSETQHKLLAEALESQTLLGPLELVGSLLEQSAPWQERSTMSLPPGLLGNSWGEGAPAWVLLDECGLELGEDTPHVCWEPQAQGRMCALYASLALLSGLSQEPH

SEQ ID NO: 4 - protein, 16 aa, synthetic construct
GVPAEGAFTEDFQGLR

SEQ ID NO: 5 - protein, 18 aa, synthetic construct
TDGVPAEGAFTEDFQGLR

SEQ ID NO: 6 - protein, 8 aa, synthetic construct
GYTFTNYW

SEQ ID NO: 7 - protein, 8 aa, synthetic construct
TKPSNGDI

SEQ ID NO: 8 - protein, 5 aa, synthetic construct
AVGYY

SEQ ID NO: 9 - protein, 12 aa, synthetic construct
QSLLNSGNQKNY

SEQ ID NO: 10 - protein, 9 aa, synthetic construct
QNDYSYPLT